European Patent Application EP 4 273 167 A1, published November 8, 2023. Title: ANTI-CLDN18.2 ANTIBODY, AND PREPARATION METHOD THEREFOR AND USE THEREOF. Applicant: Bio-Thera Solutions, Ltd. The sequence listing filed with the application follows.

SEQUENCE LISTING (108 sequences)

SEQ ID NO: 1 - protein, 120 aa, Artificial Sequence
  101VH-1
EVQLQESGPELVKPGASVKISCKASGYSFTSYYIHWVKQRPGQGLEWIGWIYPGSGNTKYNEKFKGKATLTADTSSSTAYMQLSSLTSEDSAVYYCARGMDYGNYYLDYWGQGTTLTVSS

SEQ ID NO: 2 - DNA, 360 bp, Artificial Sequence
  101VH-1
gaggtgcagctgcaggagtctggacctgagctggtgaagcctggggcttcagtgaagatatcctgcaaggcttctggctacagcttcacaagctactatatacactgggtgaagcagaggcctggacagggacttgagtggattggatggatttatcctggaagtggtaatactaagtacaatgagaagttcaagggcaaggccacactgacggcagacacatcctccagcactgcctacatgcagctcagcagcctaacatctgaggactctgcggtctattactgtgcaagggggatggactatggtaactactaccttgactactggggccaaggcaccactctcacagtctcctca

SEQ ID NO: 3 - protein, 106 aa, Artificial Sequence
  101VL-1
DIVMTQSHKFMSTSVGDRVSITCKASQDVGTAVAWYQQKPGQSPKLLIYWASTRHTGVPDRFTGSGSGTDFTLTISNVQSEDLADYFCQQYSSYLTFGAGTKLELK

SEQ ID NO: 4 - DNA, 318 bp, Artificial Sequence
  101VL-1
gacattgtgatgacccagtctcacaaattcatgtccacatcagtaggagacagggtcagcatcacctgcaaggccagtcaggatgtgggtactgctgtagcctggtatcaacagaaaccagggcaatctcctaaactactgatttactgggcatccacccggcacactggagtccctgatcgcttcacaggcagtggatctgggacagatttcactctcaccattagcaatgtgcagtctgaagacttggcagattatttctgtcagcaatatagcagctatctcacgttcggtgctgggaccaagctggagctgaaa

SEQ ID NO: 5 - protein, 107 aa, Artificial Sequence
  101VL-2
DIQLTQSPSSLSASLGDTITITCHASQNINVWLSWYQQKPGNIPKLLIYKASNLHTGVPSRFSGSGSGTGFTLTISSLQPEDIATYYCQQGQSYPYTFGGGTKLEIK

SEQ ID NO: 6 - DNA, 321 bp, Artificial Sequence
  101VL-2
gacatccagctgactcagtctccatccagtctgtctgcatcccttggagacacaattaccatcacttgccatgccagtcagaacattaatgtttggttaagctggtaccagcagaaaccaggaaatattcctaaactattgatctataaggcttccaacttgcacacaggcgtcccatcaaggtttagtggcagtggatctggaacaggtttcacattaaccatcagcagcctgcagcctgaagacattgccacttactactgtcaacagggtcaaagttatccgtacacgttcggaggggggaccaagctggaaataaaa

SEQ ID NO: 7 - protein, 119 aa, Artificial Sequence
  239VH-2
EVKLQESGGGLVKPGGSLKVSCAASGFTFSDYGMHWVRQAPEKGLEWVAYISRGRSTTYSTDTVKGRFTISRDSAKHTLFLQMTSLRSEDTAMYYCARGSYYGNAMDYWGQGTSVTVSS

SEQ ID NO: 8 - DNA, 357 bp, Artificial Sequence
  239VH-2
gaggtcaagctgcaggagtctgggggaggcttagtgaagcctggagggtccctgaaagtctcctgtgcagcctctggattcactttcagtgactatggaatgcactgggttcgtcaggctccagagaaggggctggagtgggttgcatacattagtaggggcagaagtaccacctactctacagacacagtgaagggccgattcaccatctccagagacagtgccaaacacaccctgttcctgcaaatgaccagtctgaggtctgaggacacggccatgtattactgtgcaaggggaagttactacggtaatgctatggactactggggtcaaggaacctcagtcaccgtctcctca

SEQ ID NO: 9 - protein, 122 aa, Artificial Sequence
  239VH-9
EVKLQQSVAELVRPGASVKLSCTASGFNIKNTYIYWVKQRPEQGLEWIGRIDPANGNTKYAPKFQGKATITADTSSNTAYLQLSSLTSEDTAIYYCARSPAYYINYYAMDYWGQGTSVTVSS

SEQ ID NO: 10 - DNA, 366 bp, Artificial Sequence
  239VH-9
gaggtcaagctgcagcagtctgtggcagagcttgtgaggccaggggcctcagtcaagttgtcctgcacagcttctggcttcaacattaaaaacacctatatatactgggtgaagcagaggcctgaacagggcctggagtggattggaaggattgatcctgcgaatggtaatactaaatatgccccgaagttccagggcaaggccactataactgcagacacatcctccaacacagcctacctgcagctcagcagcctgacatctgaggacactgccatctattactgtgctagatcgccggcctactatattaactactatgctatggactactggggtcaaggaacctcagtcaccgtctcctca

SEQ ID NO: 11 - protein, 106 aa, Artificial Sequence
  239VL-1
QIVLTQSPAIMSASPGEKVTMTCSASSSVSYMHWYQQKSGTSPKRWIYDTSKLASGVPARFSGSGSGTSYSLTISSMEAEDAATYYCQQWSSNPFTFGSGTKLEIK

SEQ ID NO: 12 - DNA, 318 bp, Artificial Sequence
  239VL-1
caaattgttctcacccagtctccagcaatcatgtctgcatctccaggggagaaggtcaccatgacctgcagtgccagctcaagtgtaagttacatgcactggtaccagcagaagtcaggcacctcccccaaaagatggatttatgacacatccaaactggcttctggagtccctgctcgcttcagtggcagtgggtctgggacctcttactctctcacaatcagcagcatggaggctgaagatgctgccacttattactgccagcagtggagtagtaatccattcacgttcggctcggggacaaagttggaaataaaa

SEQ ID NO: 13 - protein, 107 aa, Artificial Sequence
  239VL-4
DIVMTQSQKFMSTSVGDRVSVTCKASQNVGTNVAWYQLKPGQSPKPLIYSTSYRYSGVPDRFTGSGSGTDFTLTISNVQSEDLAEYFCQQYNSYPLTFGAGTKLELT

SEQ ID NO: 14 - DNA, 321 bp, Artificial Sequence
  239VL-4
gacattgtgatgacccagtctcagaaattcatgtccacatcagttggagacagggtcagcgtcacctgcaaggccagtcagaatgtgggtactaatgttgcctggtatcaactgaaaccagggcaatctcctaaaccactgatttactcgacatcctaccggtacagtggagtccctgatcgcttcacaggcagtggatctgggacagatttcactctcaccatcagcaatgtgcagtctgaagacttggcagagtatttctgtcagcaatataacagctatccgctcacgttcggtgctgggaccaagctggagctgaca

SEQ ID NO: 15 - protein, 113 aa, Artificial Sequence
  239VL-6
DIVMTQSPSSLTVTAGERVTMSCKSSQSLLNSGNQRNYLTWYQQKPGQPPKLLIYWASTRESGVPDRFTGSGSGTDFTLTISSVQAEDLAVYFCQSAYSYPFTFGSGTKLEIK

SEQ ID NO: 16 - DNA, 339 bp, Artificial Sequence
  239VL-6
gacattgtgatgacccagtctccatcctccctgactgtgacagcaggagagagggtcactatgagctgcaagtccagtcagagtctgttaaacagtggaaatcaaaggaactacttgacctggtaccagcagaaaccagggcagcctcctaaactgttgatctactgggcatccactagggaatctggggtccctgatcgcttcacaggcagtggatctggaacagatttcactctcaccatcagcagtgtgcaggctgaagacctggcagtctatttctgtcagagtgcttatagttatccattcacgttcggctcggggacaaagttggaaatcaaa

SEQ ID NO: 17 - protein, 119 aa, Artificial Sequence
  372VH-1
EVQLQESGGGLVKPGGSLKLSCAASGFTFSDYGMHWVRQAPEKGLEWVAYISSGRSTIYSADTVKGRFTISRDNAKNTLFLQMTSLRSEDTAMYYCARGGYYGNAMDYWGQGTSVTVSS

SEQ ID NO: 18 - DNA, 357 bp, Artificial Sequence
  372VH-1
gaggtgcagctgcaggagtctgggggaggcttagtgaagcctggagggtccctgaaactctcctgtgcagcctctggattcactttcagtgactatggaatgcactgggttcgtcaggctccagagaaggggctggagtgggttgcatacattagtagtggcagaagtaccatctactctgcagacacagtgaagggccgattcaccatctccagagacaatgccaagaacaccctgttcctgcaaatgaccagtctgaggtctgaggacacggccatgtattactgtgcaaggggaggttactacggtaatgctatggactactggggtcaaggaacctcagtcaccgtctcctca

SEQ ID NO: 19 - protein, 126 aa, Artificial Sequence
  372VH-6
EVKLQESGPELVKPGASVKMSCKASGYTFTDYYMHWVKQKPGKGLEWIGEIYPGSGNTYYNEKFKGKATLTADTSSSTAYMQLSSLTSEDSAVYFCAGGGDYYDYDGTGYYAMDYWGQGTSVTVSS

SEQ ID NO: 20 - DNA, 378 bp, Artificial Sequence
  372VH-6
gaggtgaagctgcaggagtctggacctgagctggtaaagcctggggcttcagtgaagatgtcctgcaaggcttctggatacacattcactgactactacatgcactgggtgaagcagaagcctgggaagggccttgagtggattggagagatttatcctggaagtggtaatacttactacaatgagaagttcaagggcaaggccacactgactgcagacacatcctccagcacagcctacatgcagctcagcagcctgacatctgaggactctgcagtctatttctgtgcgggggggggggactactatgattacgacgggacgggttactatgctatggactactggggtcaaggaacctcagtcaccgtctcctca

SEQ ID NO: 21 - protein, 108 aa, Artificial Sequence
  372VL-1
QIVLTQSPAIMSASPGEKVTLTCSASSSVSSSYLYWYQQKPGSSPKLWIYSTSNLASGVPARFSGSGSGTSYSLTISSMEAEDAASYFCHQWSSYPPTFGGGTKLEIK

SEQ ID NO: 22 - DNA, 324 bp, Artificial Sequence
  372VL-1
caaattgttctcacccagtctccagcaatcatgtctgcatctcctggggagaaggtcaccttgacctgcagtgccagctcaagtgtaagttccagctacttgtactggtaccagcagaagccaggatcctcccccaaactctggatttatagcacatccaacctggcttctggagtccctgctcgcttcagtggcagtgggtctgggacctcttactctctcacaatcagcagcatggaggctgaagatgctgcctcttatttctgccatcagtggagtagttacccacccacgttcggaggggggaccaagctggaaataaaa

SEQ ID NO: 23 - protein, 110 aa, Artificial Sequence
  394VH-1
EVQLQESGETVKISCKASGYIFTTSGMSWVIQAPGKGLKWMGLINTYSGVPTYADDFKGRFAFSLETSASTAYLQINNLENEDTATYFCAIWSRAWFPYWGQGTLVTVSA

SEQ ID NO: 24 - DNA, 330 bp, Artificial Sequence
  394VH-1
gaggtgcagctgcaggagtctggagagacagtcaagatctcctgcaaggcttctgggtatattttcacaacctctggaatgagttgggtgattcaggctccaggaaagggtttaaagtggatgggcttgataaacacctactctggagtgccaacatatgctgatgacttcaagggacggtttgccttctctttggaaacctctgccagcactgcctatttgcagatcaacaacctcgaaaatgaagacacggctacatatttctgtgcaatatggtcccgggcctggtttccttactggggccaagggactctggtcactgtctctgca

SEQ ID NO: 25 - protein, 121 aa, Artificial Sequence
  394VH-2
EVKLQESGAELMKPGASVKLSCKATGYTFTGYWIEWVKQRPGHGLEWIGEILPGSGSTNYNEKFKGKATFTADTSSNTAYMQLSSLTTEDSAIYYCARAPLEGLRSGFAYWGQGTLVTVSA

SEQ ID NO: 26 - DNA, 363 bp, Artificial Sequence
  394VH-2
gaggtgaagctgcaggagtctggagctgagctgatgaagcctggggcctcagtgaagctttcctgcaaggctactggctacacattcactggctactggatagagtgggtaaagcagaggcctggacatggccttgagtggattggagagattttacctggaagtggtagtactaactacaatgagaagttcaagggcaaggccacattcactgcagatacatcctccaacacagcctacatgcaactcagcagcctgacaactgaggactctgccatctattactgtgcaagagcccccttggaagggctacggagcgggtttgcttactggggccaagggactctggtcactgtctctgca

SEQ ID NO: 27 - protein, 111 aa, Artificial Sequence
  394VL-1
DIVLTQSPASLAVSLGQRATISCRASESVDSYGNSFMHWYQQKPGQPPKLLIYRASNLESGIPARFSGSGSRTDFTLTINPVEADDVATYYCQQSNEDPRTFGGGTKLEIK

SEQ ID NO: 28 - DNA, 333 bp, Artificial Sequence
  394VL-1
gacattgtgctgacccaatctccagcttctttggctgtgtctctagggcagagggccaccatatcctgcagagccagtgaaagtgttgatagttatggcaatagttttatgcactggtaccagcagaaaccaggacagccacccaaactcctcatctatcgtgcatccaacctagaatctgggatccctgccaggttcagtggcagtgggtctaggacagacttcaccctcaccattaatcctgtggaggctgatgatgttgcaacctattactgtcagcaaagtaatgaggatcctcggacgttcggtggaggcaccaagctggaaatcaaa

SEQ ID NO: 29 - protein, 107 aa, Artificial Sequence
  394VL-4
DIVMTQSPATLSVTPGDRVSLSCRASQSISDYLHWYQQKSHESPRLLIKYASQSISGIPSRFSGSGSGSDFTLSINSVEPEDVGVYYCQNGHSFPYTFGGGTKLEIK

SEQ ID NO: 30 - DNA, 321 bp, Artificial Sequence
  394VL-4
gacattgtgatgacccagtctccagccaccctgtctgtgactccaggagatagagtctctctttcctgcagggccagccagagtattagcgactacttacactggtatcaacaaaaatcacatgagtctccaaggcttctcatcaaatatgcttcccaatccatctctgggatcccctccaggttcagtggcagtggatcagggtcagatttcactctcagtatcaacagtgtggaacctgaagatgttggagtgtattactgtcaaaatggtcacagctttccgtacacgttcggaggggggaccaagctggaaataaaa

SEQ ID NO: 31 - protein, 119 aa, Artificial Sequence
  H239H-2a
EVQLLESGGGLVQPGGSLRLSCAASGFTFSDYGMHWVRQAPGKGLEWVAYISRGRSTTYSTDTVKGRFTISRDSSKNTLYLQMNSLRAEDTAVYYCARGSYYGNAMDYWGQGTLVTVSS

SEQ ID NO: 32 - DNA, 357 bp, Artificial Sequence
  H239H-2a
gaagtgcagctgctggaatcaggaggaggactggtgcagccaggaggatctctgagactgtcttgcgcagcttctggatttaccttctccgattacggcatgcattgggtgagacaggctccaggaaaaggactcgagtgggtggcttatatctctagaggaagatctaccacctactctaccgataccgtgaagggaagattcaccatctccagagactcttccaagaacaccctgtacctgcagatgaactctctgagagcagaggatacagcagtgtactattgcgctagaggctcttactacggcaacgctatggactattggggacagggaacactggtgacagtgtcttca

SEQ ID NO: 33 - protein, 119 aa, Artificial Sequence
  H239H-2b
EVQLLESGGGLVQPGGSLRLSCAASGFTFSDYGMHWVRQAPGKGLEWVAYISRGRSTTYSTDTVKGRFTISRDNSKNTLYLQMNSLRAEDTAVYYCARGSYYGNAMDYWGQGTLVTVSS

SEQ ID NO: 34 - DNA, 357 bp, Artificial Sequence
  H239H-2b
gaagtgcagctgctggaatcaggaggaggactggtgcagccaggaggatctctgagactgtcttgcgcagcttctggatttaccttctccgattacggcatgcattgggtgagacaggctccaggaaaaggactcgagtgggtggcttatatctctagaggaagatctaccacctactctaccgataccgtgaagggaagattcaccatctccagagacaactccaagaacaccctgtacctgcagatgaactctctgagagcagaggatacagcagtgtactattgcgctagaggctcttactacggcaacgctatggactattggggacagggaacactggtgacagtgtcttca

SEQ ID NO: 35 - protein, 113 aa, Artificial Sequence
  H239K-6a
DIVMTQSPDSLAVSLGERATINCKSSQSLLNSGNQRNYLTWYQQKPGQPPKLLIYWASTRESGVPDRFSGSGSGTDFTLTISSLQAEDVAVYYCQSAYSYPFTFGGGTKLEIK

SEQ ID NO: 36 - DNA, 339 bp, Artificial Sequence
  H239K-6a
gacatcgtgatgacccagtctccagattctctggcagtgtctctgggagaaagagctacaatcaactgcaagtcctctcagtctctgctgaactccggcaaccagagaaactacctgacttggtaccagcagaaaccaggacagcctcctaagctgctgatctattgggcttctaccagggaatccggagtgccagatagattttccggatctggatccggcaccgattttacactgacaatctcttctctgcaggcagaagacgtggctgtgtattattgccagtccgcctactcctacccttttacctttggcggaggaacaaagctggagatcaag

SEQ ID NO: 37 - protein, 330 aa, Artificial Sequence [sequence omitted]

SEQ ID NO: 38 - DNA, 990 bp, Artificial Sequence
  IgG1
gcttctaccaagggaccttcagtgtttcctctggctccttcttctaagtctacatccggaggaacagccgcactgggttgtctggtgaaagactacttccccgaaccggtgacggtgtcgtggaactcaggcgccctgaccagcggcgtgcacaccttcccggctgtcctacagtcctcaggactctactccctcagcagcgtggtgaccgtgccctccagcagcttgggcacccagacctacatctgcaacgtgaatcacaagcccagcaacaccaaggtggacaagaaagttgagcccaaatcttgtgacaaaactcacacatgcccaccgtgcccagcacctgaactcctggggggaccgtcagtcttcctcttccccccaaaacccaaggacaccctcatgatctcccggacccctgaggtcacatgcgtggtggtggacgtgagccacgaagaccctgaggtcaagttcaactggtacgtggacggcgtggaggtgcataatgccaagacaaagccgcgggaggagcagtacaacagcacgtaccgtgtggtcagcgtcctcaccgtcctgcaccaggactggctgaatggcaaggagtacaagtgcaaggtctccaacaaagccctcccagcccccatcgagaaaaccatctccaaagccaaagggcagccccgagaaccacaggtgtacaccctgcccccatcccgggatgagctgaccaagaaccaggtcagcctgacctgcctggtcaaaggcttctatcccagcgacatcgccgtggagtgggagagcaatgggcagccggagaacaactacaagaccacgcctcccgtgctggactccgacggctccttcttcctctacagcaagctcaccgtggacaagagcaggtggcagcaggggaacgtcttctcatgctccgtgatgcatgaggctctgcacaaccactacacgcagaagagcctctccctgtctccgggtaaa

SEQ ID NO: 39 - protein, 107 aa, Artificial Sequence [sequence omitted]

SEQ ID NO: 40 - DNA, 321 bp, Artificial Sequence
  kappa
cgtacggtggctgcaccatctgtcttcatcttcccgccatctgatgagcagttgaaatctggaactgcctctgttgtgtgcctgctgaataacttctatcccagagaggccaaagtacagtggaaggtggataacgccctccaatcgggtaactcccaggagagtgtcacagagcaggacagcaaggacagcacctacagcctcagcagcaccctgacgctgagcaaagcagactacgagaaacacaaagtctacgcctgcgaagtcacccatcagggcctgagctcgcccgtcacaaagagcttcaacaggggagagtgt

SEQ ID NO: 41 - protein, 5 aa, Artificial Sequence
  VH CDR1
SYYIH

SEQ ID NO: 42 - protein, 17 aa, Artificial Sequence
  VH CDR2
WIYPGSGNTKYNEKFKG

SEQ ID NO: 43 - protein, 11 aa, Artificial Sequence
  VH CDR3
GMDYGNYYLDY

SEQ ID NO: 44 - protein, 5 aa, Artificial Sequence
  VH CDR1
DYGMH

SEQ ID NO: 45 - protein, 17 aa, Artificial Sequence
  VH CDR2
YISRGRSTTYSTDTVKG

SEQ ID NO: 46 - protein, 10 aa, Artificial Sequence
  VH CDR3
GSYYGNAMDY

SEQ ID NO: 47 - protein, 5 aa, Artificial Sequence
  VH CDR1
NTYIY

SEQ ID NO: 48 - protein, 17 aa, Artificial Sequence
  VH CDR2
RIDPANGNTKYAPKFQG

SEQ ID NO: 49 - protein, 13 aa, Artificial Sequence
  VH CDR3
SPAYYINYYAMDY

SEQ ID NO: 50 - protein, 17 aa, Artificial Sequence
  VH CDR2
YISSGRSTIYSADTVKG

SEQ ID NO: 51 - protein, 10 aa, Artificial Sequence
  VH CDR3
GGYYGNAMDY

SEQ ID NO: 52 - protein, 5 aa, Artificial Sequence
  VH CDR1
DYYMH

SEQ ID NO: 53 - protein, 17 aa, Artificial Sequence
  VH CDR2
EIYPGSGNTYYNEKFKG

SEQ ID NO: 54 - protein, 17 aa, Artificial Sequence
  VH CDR3
GGDYYDYDGTGYYAMDY

SEQ ID NO: 55 - protein, 5 aa, Artificial Sequence
  VH CDR1
TSGMS

SEQ ID NO: 56 - protein, 17 aa, Artificial Sequence
  VH CDR2
LINTYSGVPTYADDFKG

SEQ ID NO: 57 - protein, 8 aa, Artificial Sequence
  VH CDR3
WSRAWFPY

SEQ ID NO: 58 - protein, 5 aa, Artificial Sequence
  VH CDR1
GYWIE

SEQ ID NO: 59 - protein, 17 aa, Artificial Sequence
  VH CDR2
EILPGSGSTNYNEKFKG

SEQ ID NO: 60 - protein, 12 aa, Artificial Sequence
  VH CDR3
APLEGLRSGFAY

SEQ ID NO: 61 - protein, 11 aa, Artificial Sequence
  VL CDR1
KASQDVGTAVA

SEQ ID NO: 62 - protein, 7 aa, Artificial Sequence
  VL CDR2
WASTRHT

SEQ ID NO: 63 - protein, 8 aa, Artificial Sequence
  VL CDR3
QQYSSYLT

SEQ ID NO: 64 - protein, 11 aa, Artificial Sequence
  VL CDR1
HASQNINVWLS

SEQ ID NO: 65 - protein, 7 aa, Artificial Sequence
  VL CDR2
KASNLHT

SEQ ID NO: 66 - protein, 9 aa, Artificial Sequence
  VL CDR3
QQGQSYPYT

SEQ ID NO: 67 - protein, 10 aa, Artificial Sequence
  VL CDR1
SASSSVSYMH

SEQ ID NO: 68 - protein, 7 aa, Artificial Sequence
  VL CDR2
DTSKLAS

SEQ ID NO: 69 - protein, 9 aa, Artificial Sequence
  VL CDR3
QQWSSNPFT

SEQ ID NO: 70 - protein, 11 aa, Artificial Sequence
  VL CDR1
KASQNVGTNVA

SEQ ID NO: 71 - protein, 7 aa, Artificial Sequence
  VL CDR2
STSYRYS

SEQ ID NO: 72 - protein, 9 aa, Artificial Sequence
  VL CDR3
QQYNSYPLT

SEQ ID NO: 73 - protein, 17 aa, Artificial Sequence
  VL CDR1
KSSQSLLNSGNQRNYLT

SEQ ID NO: 74 - protein, 7 aa, Artificial Sequence
  VL CDR2
WASTRES

SEQ ID NO: 75 - protein, 9 aa, Artificial Sequence
  VL CDR3
QSAYSYPFT

SEQ ID NO: 76 - protein, 12 aa, Artificial Sequence
  VL CDR1
SASSSVSSSYLY

SEQ ID NO: 77 - protein, 7 aa, Artificial Sequence
  VL CDR2
STSNLAS

SEQ ID NO: 78 - protein, 9 aa, Artificial Sequence
  VL CDR3
HQWSSYPPT

SEQ ID NO: 79 - protein, 15 aa, Artificial Sequence
  VL CDR1
RASESVDSYGNSFMH

SEQ ID NO: 80 - protein, 7 aa, Artificial Sequence
  VL CDR2
RASNLES

SEQ ID NO: 81 - protein, 9 aa, Artificial Sequence
  VL CDR3
QQSNEDPRT

SEQ ID NO: 82 - protein, 11 aa, Artificial Sequence
  VL CDR1
RASQSISDYLH

SEQ ID NO: 83 - protein, 7 aa, Artificial Sequence
  VL CDR2
YASQSIS

SEQ ID NO: 84 - protein, 9 aa, Artificial Sequence
  VL CDR3
QNGHSFPYT

SEQ ID NO: 85 - DNA, 6 bp, Artificial Sequence
  5’HindIII
aagctt

SEQ ID NO: 86 - DNA, 6 bp, Artificial Sequence
  3’BsiWI
cgtacg

SEQ ID NO: 87 - DNA, 6 bp, Artificial Sequence
  3’ AgeI
accggt

SEQ ID NO: 88 - DNA, 9 bp, Artificial Sequence
  kozak
gccgccacc

SEQ ID NO: 89 - protein, 22 aa, Artificial Sequence
  Light chain Signal peptide
MDMRVLAQLLGLLLLCFPGARC

SEQ ID NO: 90 - DNA, 66 bp, Artificial Sequence
  Light chain Signal peptide
atggacatgagggtgctggcccagctgctgggactgctgctgctgtgcttcccaggcgccagatgc

SEQ ID NO: 91 - protein, 19 aa, Artificial Sequence
  Heavy chain Signal peptide
MGWSLILLFLVAVATRVLS

SEQ ID NO: 92 - DNA, 57 bp, Artificial Sequence
  Heavy chain Signal peptide
atgggttggtctctgattctcctgtttctggtggcagtggctacaagagtcctgtca

SEQ ID NO: 93 - protein, 261 aa, Artificial Sequence
  The full-length amino acid sequence of human CLDN18.2
MAVTACQGLGFVVSLIGIAGIIAATCMDQWSTQDLYNNPVTAVFNYQGLWRSCVRESSGFTECRGYFTLLGLPAMLQAVRALMIVGIVLGAIGLLVSIFALKCIRIGSMEDSAKANMTLTSGIMFIVSGLCAIAGVSVFANMLVTNFWMSTANMYTGMGGMVQTVQTRYTFGAALFVGWVAGGLTLIGGVMMCIACRGLAPEETNYKAVSYHASGHSVAYKPGGFKASTGFGSNTKNKKIYDGGARTEDEVQSYPSKHDYV

SEQ ID NO: 94 - DNA, 783 bp, Artificial Sequence
  The corresponding nucleic acid sequence of human CLDN18.2
atggccgtgactgcctgtcagggcttggggttcgtggtttcactgattgggattgcgggcatcattgctgccacctgcatggaccagtggagcacccaagacttgtacaacaaccccgtaacagctgttttcaactaccaggggctgtggcgctcctgtgtccgagagagctctggcttcaccgagtgccggggctacttcaccctgctggggctgccagccatgctgcaggcagtgcgagccctgatgatcgtaggcatcgtcctgggtgccattggcctcctggtatccatctttgccctgaaatgcatccgcattggcagcatggaggactctgccaaagccaacatgacactgacctccgggatcatgttcattgtctcaggtctttgtgcaattgctggagtgtctgtgtttgccaacatgctggtgactaacttctggatgtccacagctaacatgtacaccggcatgggtgggatggtgcagactgttcagaccaggtacacatttggtgcggctctgttcgtgggctgggtcgctggaggcctcacactaattgggggtgtgatgatgtgcatcgcctgccggggcctggcaccagaagaaaccaactacaaagccgtttcttatcatgcctcaggccacagtgttgcctacaagcctggaggcttcaaggccagcactggctttgggtccaacaccaaaaacaagaagatatacgatggaggtgcccgcacagaggacgaggtacaatcttatccttccaagcacgactatgtg

SEQ ID NO: 95 - protein, 261 aa, Artificial Sequence
  The full-length amino acid sequence of human CLDN18.1
MSTTTCQVVAFLLSILGLAGCIAATGMDMWSTQDLYDNPVTSVFQYEGLWRSCVRQSSGFTECRPYFTILGLPAMLQAVRALMIVGIVLGAIGLLVSIFALKCIRIGSMEDSAKANMTLTSGIMFIVSGLCAIAGVSVFANMLVTNFWMSTANMYTGMGGMVQTVQTRYTFGAALFVGWVAGGLTLIGGVMMCIACRGLAPEETNYKAVSYHASGHSVAYKPGGFKASTGFGSNTKNKKIYDGGARTEDEVQSYPSKHDYV

SEQ ID NO: 96 - DNA, 783 bp, Artificial Sequence
  The corresponding nucleic acid sequence of human CLDN18.1
atgtccaccaccacatgccaagtggtggcgttcctcctgtccatcctggggctggccggctgcatcgcggccaccgggatggacatgtggagcacccaggacctgtacgacaaccccgtcacctccgtgttccagtacgaagggctctggaggagctgcgtgaggcagagttcaggcttcaccgaatgcaggccctatttcaccatcctgggacttccagccatgctgcaggcagtgcgagccctgatgatcgtaggcatcgtcctgggtgccattggcctcctggtatccatctttgccctgaaatgcatccgcattggcagcatggaggactctgccaaagccaacatgacactgacctccgggatcatgttcattgtctcaggtctttgtgcaattgctggagtgtctgtgtttgccaacatgctggtgactaacttctggatgtccacagctaacatgtacaccggcatgggtgggatggtgcagactgttcagaccaggtacacatttggtgcggctctgttcgtgggctgggtcgctggaggcctcacactaattgggggtgtgatgatgtgcatcgcctgccggggcctggcaccagaagaaaccaactacaaagccgtttcttatcatgcctcaggccacagtgttgcctacaagcctggaggcttcaaggccagcactggctttgggtccaacaccaaaaacaagaagatatacgatggaggtgcccgcacagaggacgaggtacaatcttatccttccaagcacgactatgtg

SEQ ID NO: 97 - DNA, 23 bp, Artificial Sequence
  VhRevU
gaggtsmarctgcagsagtcwgg

SEQ ID NO: 98 - DNA, 20 bp, Artificial Sequence
  VhForU
gacagtggataracmgatgg

SEQ ID NO: 99 - DNA, 23 bp, Artificial Sequence
  VkRev1
gaggtsmarctgcagsagtcwgg

SEQ ID NO: 100 - DNA, 21 bp, Artificial Sequence
  VkRev2
gatattgtgatgacgcaggct

SEQ ID NO: 101 - DNA, 18 bp, Artificial Sequence
  VkRev3
gatattgtgataacccag

SEQ ID NO: 102 - DNA, 21 bp, Artificial Sequence
  VkRev4
gacattgtgctgacccaatct

SEQ ID NO: 103 - DNA, 21 bp, Artificial Sequence
  VkRev5
gacattgtgatgacccagtct

SEQ ID NO: 104 - DNA, 21 bp, Artificial Sequence
  VkRev6
gatattgtgctaactcagtct

SEQ ID NO: 105 - DNA, 21 bp, Artificial Sequence
  VkRev7
gatatccagatgacacagact

SEQ ID NO: 106 - DNA, 21 bp, Artificial Sequence
  VkRev8
gacatccagctgactcagtct

SEQ ID NO: 107 - DNA, 21 bp, Artificial Sequence
  VkRev9
caaattgttctcacccagtct

SEQ ID NO: 108 - DNA, 21 bp, Artificial Sequence
  VkForU
ggatacagttggtgcagcatc